European Patent Specification EP 3 209 681 B1, published April 2, 2025. Title: Pharmaceutical Compositions Comprising Peptide Variants and Methods of Use Thereof. Applicant: NGM Biopharmaceuticals, Inc. LINDHOUT, Darrin Anthony OLSON, Charles. The sequence listing filed with the application follows.

SEQUENCE LISTING (205 sequences)

SEQ ID NO: 1 - protein, 194 aa, Homo sapiens
RPLAFSDASPHVHYGWGDPIRLRHLYTSGPHGLSSCFLRIRADGVVDCARGQSAHSLLEIKAVALRTVAIKGVHSVRYLCMGADGKMQGLLQYSEEDCAFEEEIRPDGYNVYRSEKHRLPVSLSSAKQRQLYKNRGFLPLSHFLPMLPMVPEEPEDLRGHLESDMFSSPLETDSMDPFGLVTGLEAVRSPSFEK

SEQ ID NO: 2 - protein, 194 aa, Homo sapiens
RPLAFSDSSPLVHYGWGDPIRLRHLYTSGPHGLSSCFLRIRADGVVDCARGQSAHSLLEIKAVALRTVAIKGVHSVRYLCMGADGKMQGLLQYSEEDCAFEEEIRPDGYNVYRSEKHRLPVSLSSAKQRQLYKNRGFLPLSHFLPMLPMVPEEPEDLRGHLESDMFSSPLETDSMDPFGLVTGLEAVRSPSFEK

SEQ ID NO: 3 - protein, 194 aa, Homo sapiens
RPLAFSDAGPHVHYGWGDPIRLRHLYTSGPHGLSSCFLRIRADGVVDCARGQSAHSLLEIKAVALRTVAIKGVHSVRYLCMGADGKMQGLLQYSEEDCAFEEEILEDGYNVYRSEKHRLPVSLSSAKQRQLYKNRGFLPLSHFLPMLPMVPEEPEDLRGHLESDMFSSPLETDSMDPFGLVTGLEAVRSPSFEK

SEQ ID NO: 4 - protein, 194 aa, Homo sapiens
RPLAFSDAGPHVHYAWGDPIRLRHLYTSGPHGLSSCFLRIRADGVVDCARGQSAHSLLEIKAVALRTVAIKGVHSVRYLCMGADGKMQGLLQYSEEDCAFEEEIRPDGYNVYRSEKHRLPVSLSSAKQRQLYKNRGFLPLSHFLPMLPMVPEEPEDLRGHLESDMFSSPLETDSMDPFGLVTGLEAVRSPSFEK

SEQ ID NO: 5 - protein, 191 aa, Homo sapiens
RHPIPDSSPLLQFGGQVRLRHLYTSGPHGLSSCFLRIRADGVVDCARGQSAHSLLEIKAVALRTVAIKGVHSVRYLCMGADGKMQGLLQYSEEDCAFEEEIRPDGYNVYRSEKHRLPVSLSSAKQRQLYKNRGFLPLSHFLPMLPMVPEEPEDLRGHLESDMFSSPLETDSMDPFGLVTGLEAVRSPSFEK

SEQ ID NO: 6 - protein, 187 aa, Homo sapiens
RDSSPLLQFGGQVRLRHLYTSGPHGLSSCFLRIRADGVVDCARGQSAHSLLEIKAVALRTVAIKGVHSVRYLCMGADGKMQGLLQYSEEDCAFEEEIRPDGYNVYRSEKHRLPVSLSSAKQRQLYKNRGFLPLSHFLPMLPMVPEEPEDLRGHLESDMFSSPLETDSMDPFGLVTGLEAVRSPSFEK

SEQ ID NO: 7 - protein, 192 aa, Homo sapiens
RPLAFSDSSPLLQFGGQVRLRHLYTSGPHGLSSCFLRIRADGVVDCARGQSAHSLLEIKAVALRTVAIKGVHSVRYLCMGADGKMQGLLQYSEEDCAFEEEIRPDGYNVYRSEKHRLPVSLSSAKQRQLYKNRGFLPLSHFLPMLPMVPEEPEDLRGHLESDMFSSPLETDSMDPFGLVTGLEAVRSPSFEK

SEQ ID NO: 8 - protein, 191 aa, Homo sapiens
RHPIPDSSPLLQWGDPIRLRHLYTSGPHGLSSCFLRIRADGVVDCARGQSAHSLLEIKAVALRTVAIKGVHSVRYLCMGADGKMQGLLQYSEEDCAFEEEIRPDGYNVYRSEKHRLPVSLSSAKQRQLYKNRGFLPLSHFLPMLPMVPEEPEDLRGHLESDMFSSPLETDSMDPFGLVTGLEAVRSPSFEK

SEQ ID NO: 9 - protein, 193 aa, Homo sapiens
RHPIPDSSPLLQFGWGDPIRLRHLYTSGPHGLSSCFLRIRADGVVDCARGQSAHSLLEIKAVALRTVAIKGVHSVRYLCMGADGKMQGLLQYSEEDCAFEEEIRPDGYNVYRSEKHRLPVSLSSAKQRQLYKNRGFLPLSHFLPMLPMVPEEPEDLRGHLESDMFSSPLETDSMDPFGLVTGLEAVRSPSFEK

SEQ ID NO: 10 - protein, 193 aa, Homo sapiens
RHPIPDSSPHVHYGWGDPIRLRHLYTSGPHGLSSCFLRIRADGVVDCARGQSAHSLLEIKAVALRTVAIKGVHSVRYLCMGADGKMQGLLQYSEEDCAFEEEIRPDGYNVYRSEKHRLPVSLSSAKQRQLYKNRGFLPLSHFLPMLPMVPEEPEDLRGHLESDMFSSPLETDSMDPFGLVTGLEAVRSPSFEK

SEQ ID NO: 11 - protein, 192 aa, Homo sapiens
RPLAFSDAGPLLQWGDPIRLRHLYTSGPHGLSSCFLRIRADGVVDCARGQSAHSLLEIKAVALRTVAIKGVHSVRYLCMGADGKMQGLLQYSEEDCAFEEEIRPDGYNVYRSEKHRLPVSLSSAKQRQLYKNRGFLPLSHFLPMLPMVPEEPEDLRGHLESDMFSSPLETDSMDPFGLVTGLEAVRSPSFEK

SEQ ID NO: 12 - protein, 194 aa, Homo sapiens
RPLAFSDAGPLLQFGWGDPIRLRHLYTSGPHGLSSCFLRIRADGVVDCARGQSAHSLLEIKAVALRTVAIKGVHSVRYLCMGADGKMQGLLQYSEEDCAFEEEIRPDGYNVYRSEKHRLPVSLSSAKQRQLYKNRGFLPLSHFLPMLPMVPEEPEDLRGHLESDMFSSPLETDSMDPFGLVTGLEAVRSPSFEK

SEQ ID NO: 13 - protein, 192 aa, Homo sapiens
RPLAFSDAGPLLQFGGQVRLRHLYTSGPHGLSSCFLRIRADGVVDCARGQSAHSLLEIKAVALRTVAIKGVHSVRYLCMGADGKMQGLLQYSEEDCAFEEEIRPDGYNVYRSEKHRLPVSLSSAKQRQLYKNRGFLPLSHFLPMLPMVPEEPEDLRGHLESDMFSSPLETDSMDPFGLVTGLEAVRSPSFEK

SEQ ID NO: 14 - protein, 191 aa, Homo sapiens
RHPIPDSSPHVHYGGQVRLRHLYTSGPHGLSSCFLRIRADGVVDCARGQSAHSLLEIKAVALRTVAIKGVHSVRYLCMGADGKMQGLLQYSEEDCAFEEEIRPDGYNVYRSEKHRLPVSLSSAKQRQLYKNRGFLPLSHFLPMLPMVPEEPEDLRGHLESDMFSSPLETDSMDPFGLVTGLEAVRSPSFEK

SEQ ID NO: 15 - protein, 192 aa, Homo sapiens
RPLAFSDAGPHVHYGGQVRLRHLYTSGPHGLSSCFLRIRADGVVDCARGQSAHSLLEIKAVALRTVAIKGVHSVRYLCMGADGKMQGLLQYSEEDCAFEEEIRPDGYNVYRSEKHRLPVSLSSAKQRQLYKNRGFLPLSHFLPMLPMVPEEPEDLRGHLESDMFSSPLETDSMDPFGLVTGLEAVRSPSFEK

SEQ ID NO: 16 - protein, 192 aa, Homo sapiens
RPLAFSDAGPHVHWGDPIRLRHLYTSGPHGLSSCFLRIRADGVVDCARGQSAHSLLEIKAVALRTVAIKGVHSVRYLCMGADGKMQGLLQYSEEDCAFEEEIRPDGYNVYRSEKHRLPVSLSSAKQRQLYKNRGFLPLSHFLPMLPMVPEEPEDLRGHLESDMFSSPLETDSMDPFGLVTGLEAVRSPSFEK

SEQ ID NO: 17 - protein, 192 aa, Homo sapiens
RPLAFSDAGPHVGWGDPIRLRHLYTSGPHGLSSCFLRIRADGVVDCARGQSAHSLLEIKAVALRTVAIKGVHSVRYLCMGADGKMQGLLQYSEEDCAFEEEIRPDGYNVYRSEKHRLPVSLSSAKQRQLYKNRGFLPLSHFLPMLPMVPEEPEDLRGHLESDMFSSPLETDSMDPFGLVTGLEAVRSPSFEK

SEQ ID NO: 18 - protein, 192 aa, Homo sapiens
RPLAFSDAGPHYGWGDPIRLRHLYTSGPHGLSSCFLRIRADGVVDCARGQSAHSLLEIKAVALRTVAIKGVHSVRYLCMGADGKMQGLLQYSEEDCAFEEEIRPDGYNVYRSEKHRLPVSLSSAKQRQLYKNRGFLPLSHFLPMLPMVPEEPEDLRGHLESDMFSSPLETDSMDPFGLVTGLEAVRSPSFEK

SEQ ID NO: 19 - protein, 192 aa, Homo sapiens
RPLAFSDAGPVYGWGDPIRLRHLYTSGPHGLSSCFLRIRADGVVDCARGQSAHSLLEIKAVALRTVAIKGVHSVRYLCMGADGKMQGLLQYSEEDCAFEEEIRPDGYNVYRSEKHRLPVSLSSAKQRQLYKNRGFLPLSHFLPMLPMVPEEPEDLRGHLESDMFSSPLETDSMDPFGLVTGLEAVRSPSFEK

SEQ ID NO: 20 - protein, 192 aa, Homo sapiens
RPLAFSDAGPVHGWGDPIRLRHLYTSGPHGLSSCFLRIRADGVVDCARGQSAHSLLEIKAVALRTVAIKGVHSVRYLCMGADGKMQGLLQYSEEDCAFEEEIRPDGYNVYRSEKHRLPVSLSSAKQRQLYKNRGFLPLSHFLPMLPMVPEEPEDLRGHLESDMFSSPLETDSMDPFGLVTGLEAVRSPSFEK

SEQ ID NO: 21 - protein, 192 aa, Homo sapiens
RPLAFSDAGPVHYWGDPIRLRHLYTSGPHGLSSCFLRIRADGVVDCARGQSAHSLLEIKAVALRTVAIKGVHSVRYLCMGADGKMQGLLQYSEEDCAFEEEIRPDGYNVYRSEKHRLPVSLSSAKQRQLYKNRGFLPLSHFLPMLPMVPEEPEDLRGHLESDMFSSPLETDSMDPFGLVTGLEAVRSPSFEK

SEQ ID NO: 22 - protein, 193 aa, Homo sapiens
RPLAFSDAGPHVHGWGDPIRLRHLYTSGPHGLSSCFLRIRADGVVDCARGQSAHSLLEIKAVALRTVAIKGVHSVRYLCMGADGKMQGLLQYSEEDCAFEEEIRPDGYNVYRSEKHRLPVSLSSAKQRQLYKNRGFLPLSHFLPMLPMVPEEPEDLRGHLESDMFSSPLETDSMDPFGLVTGLEAVRSPSFEK

SEQ ID NO: 23 - protein, 192 aa, Homo sapiens
RPLAFSDAGPHHGWGDPIRLRHLYTSGPHGLSSCFLRIRADGVVDCARGQSAHSLLEIKAVALRTVAIKGVHSVRYLCMGADGKMQGLLQYSEEDCAFEEEIRPDGYNVYRSEKHRLPVSLSSAKQRQLYKNRGFLPLSHFLPMLPMVPEEPEDLRGHLESDMFSSPLETDSMDPFGLVTGLEAVRSPSFEK

SEQ ID NO: 24 - protein, 192 aa, Homo sapiens
RPLAFSDAGPHHYWGDPIRLRHLYTSGPHGLSSCFLRIRADGVVDCARGQSAHSLLEIKAVALRTVAIKGVHSVRYLCMGADGKMQGLLQYSEEDCAFEEEIRPDGYNVYRSEKHRLPVSLSSAKQRQLYKNRGFLPLSHFLPMLPMVPEEPEDLRGHLESDMFSSPLETDSMDPFGLVTGLEAVRSPSFEK

SEQ ID NO: 25 - protein, 192 aa, Homo sapiens
RPLAFSDAGPHVYWGDPIRLRHLYTSGPHGLSSCFLRIRADGVVDCARGQSAHSLLEIKAVALRTVAIKGVHSVRYLCMGADGKMQGLLQYSEEDCAFEEEIRPDGYNVYRSEKHRLPVSLSSAKQRQLYKNRGFLPLSHFLPMLPMVPEEPEDLRGHLESDMFSSPLETDSMDPFGLVTGLEAVRSPSFEK

SEQ ID NO: 26 - protein, 192 aa, Homo sapiens
RPLAFSDSSPLVHWGDPIRLRHLYTSGPHGLSSCFLRIRADGVVDCARGQSAHSLLEIKAVALRTVAIKGVHSVRYLCMGADGKMQGLLQYSEEDCAFEEEIRPDGYNVYRSEKHRLPVSLSSAKQRQLYKNRGFLPLSHFLPMLPMVPEEPEDLRGHLESDMFSSPLETDSMDPFGLVTGLEAVRSPSFEK

SEQ ID NO: 27 - protein, 192 aa, Homo sapiens
RPLAFSDSSPHVHWGDPIRLRHLYTSGPHGLSSCFLRIRADGVVDCARGQSAHSLLEIKAVALRTVAIKGVHSVRYLCMGADGKMQGLLQYSEEDCAFEEEIRPDGYNVYRSEKHRLPVSLSSAKQRQLYKNRGFLPLSHFLPMLPMVPEEPEDLRGHLESDMFSSPLETDSMDPFGLVTGLEAVRSPSFEK

SEQ ID NO: 28 - protein, 191 aa, Homo sapiens
RPLAFSDAGPHVWGDPIRLRHLYTSGPHGLSSCFLRIRADGVVDCARGQSAHSLLEIKAVALRTVAIKGVHSVRYLCMGADGKMQGLLQYSEEDCAFEEEIRPDGYNVYRSEKHRLPVSLSSAKQRQLYKNRGFLPLSHFLPMLPMVPEEPEDLRGHLESDMFSSPLETDSMDPFGLVTGLEAVRSPSFEK

SEQ ID NO: 29 - protein, 193 aa, Homo sapiens
RPLAFSDAGPHVHYWGDPIRLRHLYTSGPHGLSSCFLRIRADGVVDCARGQSAHSLLEIKAVALRTVAIKGVHSVRYLCMGADGKMQGLLQYSEEDCAFEEEIRPDGYNVYRSEKHRLPVSLSSAKQRQLYKNRGFLPLSHFLPMLPMVPEEPEDLRGHLESDMFSSPLETDSMDPFGLVTGLEAVRSPSFEK

SEQ ID NO: 30 - protein, 194 aa, Homo sapiens; identical to SEQ ID NO: 4

SEQ ID NO: 31 - protein, 191 aa, Homo sapiens
RHPIPDSSPLLQFGAQVRLRHLYTSGPHGLSSCFLRIRADGVVDCARGQSAHSLLEIKAVALRTVAIKGVHSVRYLCMGADGKMQGLLQYSEEDCAFEEEIRPDGYNVYRSEKHRLPVSLSSAKQRQLYKNRGFLPLSHFLPMLPMVPEEPEDLRGHLESDMFSSPLETDSMDPFGLVTGLEAVRSPSFEK

SEQ ID NO: 32 - protein, 191 aa, Homo sapiens
RHPIPDSSPLLQFGDQVRLRHLYTSGPHGLSSCFLRIRADGVVDCARGQSAHSLLEIKAVALRTVAIKGVHSVRYLCMGADGKMQGLLQYSEEDCAFEEEIRPDGYNVYRSEKHRLPVSLSSAKQRQLYKNRGFLPLSHFLPMLPMVPEEPEDLRGHLESDMFSSPLETDSMDPFGLVTGLEAVRSPSFEK

SEQ ID NO: 33 - protein, 191 aa, Homo sapiens
RHPIPDSSPLLQFGPQVRLRHLYTSGPHGLSSCFLRIRADGVVDCARGQSAHSLLEIKAVALRTVAIKGVHSVRYLCMGADGKMQGLLQYSEEDCAFEEEIRPDGYNVYRSEKHRLPVSLSSAKQRQLYKNRGFLPLSHFLPMLPMVPEEPEDLRGHLESDMFSSPLETDSMDPFGLVTGLEAVRSPSFEK

SEQ ID NO: 34 - protein, 191 aa, Homo sapiens
RHPIPDSSPLLQFGGAVRLRHLYTSGPHGLSSCFLRIRADGVVDCARGQSAHSLLEIKAVALRTVAIKGVHSVRYLCMGADGKMQGLLQYSEEDCAFEEEIRPDGYNVYRSEKHRLPVSLSSAKQRQLYKNRGFLPLSHFLPMLPMVPEEPEDLRGHLESDMFSSPLETDSMDPFGLVTGLEAVRSPSFEK

SEQ ID NO: 35 - protein, 191 aa, Homo sapiens
RHPIPDSSPLLQFGGEVRLRHLYTSGPHGLSSCFLRIRADGVVDCARGQSAHSLLEIKAVALRTVAIKGVHSVRYLCMGADGKMQGLLQYSEEDCAFEEEIRPDGYNVYRSEKHRLPVSLSSAKQRQLYKNRGFLPLSHFLPMLPMVPEEPEDLRGHLESDMFSSPLETDSMDPFGLVTGLEAVRSPSFEK

SEQ ID NO: 36 - protein, 191 aa, Homo sapiens
RHPIPDSSPLLQFGGNVRLRHLYTSGPHGLSSCFLRIRADGVVDCARGQSAHSLLEIKAVALRTVAIKGVHSVRYLCMGADGKMQGLLQYSEEDCAFEEEIRPDGYNVYRSEKHRLPVSLSSAKQRQLYKNRGFLPLSHFLPMLPMVPEEPEDLRGHLESDMFSSPLETDSMDPFGLVTGLEAVRSPSFEK

SEQ ID NO: 37 - protein, 191 aa, Homo sapiens
RHPIPDSSPLLQFGGQARLRHLYTSGPHGLSSCFLRIRADGVVDCARGQSAHSLLEIKAVALRTVAIKGVHSVRYLCMGADGKMQGLLQYSEEDCAFEEEIRPDGYNVYRSEKHRLPVSLSSAKQRQLYKNRGFLPLSHFLPMLPMVPEEPEDLRGHLESDMFSSPLETDSMDPFGLVTGLEAVRSPSFEK

SEQ ID NO: 38 - protein, 191 aa, Homo sapiens
RHPIPDSSPLLQFGGQIRLRHLYTSGPHGLSSCFLRIRADGVVDCARGQSAHSLLEIKAVALRTVAIKGVHSVRYLCMGADGKMQGLLQYSEEDCAFEEEIRPDGYNVYRSEKHRLPVSLSSAKQRQLYKNRGFLPLSHFLPMLPMVPEEPEDLRGHLESDMFSSPLETDSMDPFGLVTGLEAVRSPSFEK

SEQ ID NO: 39 - protein, 191 aa, Homo sapiens
RHPIPDSSPLLQFGGQTRLRHLYTSGPHGLSSCFLRIRADGVVDCARGQSAHSLLEIKAVALRTVAIKGVHSVRYLCMGADGKMQGLLQYSEEDCAFEEEIRPDGYNVYRSEKHRLPVSLSSAKQRQLYKNRGFLPLSHFLPMLPMVPEEPEDLRGHLESDMFSSPLETDSMDPFGLVTGLEAVRSPSFEK

SEQ ID NO: 40 - protein, 193 aa, Homo sapiens
RHPIPDSSPLLQFGWGQPVRLRHLYTSGPHGLSSCFLRIRADGVVDCARGQSAHSLLEIKAVALRTVAIKGVHSVRYLCMGADGKMQGLLQYSEEDCAFEEEIRPDGYNVYRSEKHRLPVSLSSAKQRQLYKNRGFLPLSHFLPMLPMVPEEPEDLRGHLESDMFSSPLETDSMDPFGLVTGLEAVRSPSFEK

SEQ ID NO: 41 - protein, 182 aa, Homo sapiens
RPLAFSDAGPHVHYGWGDPIRLRHLYTSGPHGLSSCFLRIRADGVVDCARGQSAHSLLEIKAVALRTVAIKGVHSVRYLCMGADGKMQGLLQYSEEDCAFEEEIRPDGYNVYRSEKHRLPVSLSSAKQRQLYKNRGFLPLSHFLPMLPEPPGILAPQPPDVGSSDPLSMVGPSQGRSPSYAS

SEQ ID NO: 42 - protein, 178 aa, Homo sapiens
HPIPDSSPLLQFGGQVRLRHLYTSGPHGLSSCFLRIRADGVVDCARGQSAHSLLEIKAVALRTVAIKGVHSVRYLCMGADGKMQGLLQYSEEDCAFEEEIRPDGYNVYRSEKHRLPVSLSSAKQRQLYKNRGFLPLSHFLPMLPEPPGILAPQPPDVGSSDPLSMVGPSQGRSPSYAS

SEQ ID NO: 43 - protein, 192 aa, Homo sapiens
RPLAFSDAGPHVHYGGDIRLRHLYTSGPHGLSSCFLRIRADGVVDCARGQSAHSLLEIKAVALRTVAIKGVHSVRYLCMGADGKMQGLLQYSEEDCAFEEEIRPDGYNVYRSEKHRLPVSLSSAKQRQLYKNRGFLPLSHFLPMLPMVPEEPEDLRGHLESDMFSSPLETDSMDPFGLVTGLEAVRSPSFEK

SEQ ID NO: 44 - protein, 185 aa, Homo sapiens
RPLAFSDAGPHVHYGWGDPIRQRYLYTDDAQQTEAHLEIREDGTVGGAADQSPESLLQLKALKPGVIQILGVKTSRFLCQRPDGALYGSLHFDPEACSFRELLLEDGYNVYQSEAHGLPLHLPGNKSPHRDPAPRGPARFLPLPGLPPALPEPPGILAPQPPDVGSSDPLSMVGPSQGRSPSYAS

SEQ ID NO: 45 - protein, 193 aa, Homo sapiens
HPIPDSSPLLQFGGQVRQRYLYTDDAQQTEAHLEIREDGTVGGAADQSPESLLQLKALKPGVIQILGVKTSRFLCQRPDGALYGSLHFDPEACSFRELLLEDGYNVYQSEAHGLPLHLPGNKSPHRDPAPRGPARFLPLPGLPPALPMVPEEPEDLRGHLESDMFSSPLETDSMDPFGLVTGLEAVRSPSFEK

SEQ ID NO: 46 - protein, 232 aa, Homo sapiens
RPLAFSDAGPHVHYGWGDPIRQRYLYTDDAQQTEAHLEIREDGTVGGAADQSPESLLQLKALKPGVIQILGVKTSRFLCQRPDGALYGSLHFDPEACSFRELLLEDGYNVYQSEAHGLPLHLPGNKSPHRDPAPRGPARFLPLPGLPPALPEPPGILAPQPPDVGSSDPLSMVGPSQGRSPSYASPMVPEEPEDLRGHLESDMFSSPLETDSMDPFGLVTGLEAVRSPSFEK

SEQ ID NO: 47 - protein, 190 aa, Homo sapiens
HPIPDSSPLLQWGDPIRLRHLYTSGPHGLSSCFLRIRADGVVDCARGQSAHSLLEIKAVALRTVAIKGVHSVRYLCMGADGKMQGLLQYSEEDCAFEEEIRPDGYNVYRSEKHRLPVSLSSAKQRQLYKNRGFLPLSHFLPMLPMVPEEPEDLRGHLESDMFSSPLETDSMDPFGLVTGLEAVRSPSFEK

SEQ ID NO: 48 - protein, 187 aa, Homo sapiens; identical to SEQ ID NO: 6

SEQ ID NO: 49 - protein, 192 aa, Homo sapiens; identical to SEQ ID NO: 7

SEQ ID NO: 50 - protein, 191 aa, Homo sapiens
RHPIPDSSPLLQFGDQVRLRHLYTSGPHGLSSCFLRIRADGVVDCARGQSAHSLLEIKAVALRTVAIKGVHSVRYLCMGADGKMQGLLQYSEEDCAFEEEILEDGYNVYRSEKHRLPVSLSSAKQRQLYKNRGFLPLSHFLPMLPMVPEEPEDLRGHLESDMFSSPLETDSMDPFGLVTGLEAVRSPSFEK

SEQ ID NO: 51 - protein, 191 aa, Homo sapiens; identical to SEQ ID NO: 36

SEQ ID NO: 52 - protein, 187 aa, Homo sapiens
RDSSPLLQWGDPIRLRHLYTSGPHGLSSCFLRIRADGVVDCARGQSAHSLLEIKAVALRTVAIKGVHSVRYLCMGADGKMQGLLQYSEEDCAFEEEIRPDGYNVYRSEKHRLPVSLSSAKQRQLYKNRGFLPLSHFLPMLPMVPEEPEDLRGHLESDMFSSPLETDSMDPFGLVTGLEAVRSPSFEK

SEQ ID NO: 53 - protein, 189 aa, Homo sapiens
MDSSPLVHYGWGDPIRLRHLYTSGPHGLSSCFLRIRADGVVDCARGQSAHSLLEIKAVALRTVAIKGVHSVRYLCMGADGKMQGLLQYSEEDCAFEEEIRPDGYNVYRSEKHRLPVSLSSAKQRQLYKNRGFLPLSHFLPMLPMVPEEPEDLRGHLESDMFSSPLETDSMDPFGLVTGLEAVRSPSFEK

SEQ ID NO: 54 - protein, 192 aa, Homo sapiens; identical to SEQ ID NO: 11

SEQ ID NO: 55 - protein, 192 aa, Homo sapiens; identical to SEQ ID NO: 18

SEQ ID NO: 56 - protein, 192 aa, Homo sapiens; identical to SEQ ID NO: 19

SEQ ID NO: 57 - protein, 192 aa, Homo sapiens; identical to SEQ ID NO: 20

SEQ ID NO: 58 - protein, 192 aa, Homo sapiens; identical to SEQ ID NO: 21

SEQ ID NO: 59 - protein, 192 aa, Homo sapiens; identical to SEQ ID NO: 23

SEQ ID NO: 60 - protein, 192 aa, Homo sapiens; identical to SEQ ID NO: 24

SEQ ID NO: 61 - protein, 192 aa, Homo sapiens; identical to SEQ ID NO: 17

SEQ ID NO: 62 - protein, 192 aa, Homo sapiens; identical to SEQ ID NO: 25

SEQ ID NO: 63 - protein, 192 aa, Homo sapiens; identical to SEQ ID NO: 16

SEQ ID NO: 64 - protein, 192 aa, Homo sapiens; identical to SEQ ID NO: 26

SEQ ID NO: 65 - protein, 192 aa, Homo sapiens; identical to SEQ ID NO: 27

SEQ ID NO: 66 - protein, 192 aa, Homo sapiens
RPLAFSDAGPHLQWGDPIRLRHLYTSGPHGLSSCFLRIRADGVVDCARGQSAHSLLEIKAVALRTVAIKGVHSVRYLCMGADGKMQGLLQYSEEDCAFEEEIRPDGYNVYRSEKHRLPVSLSSAKQRQLYKNRGFLPLSHFLPMLPMVPEEPEDLRGHLESDMFSSPLETDSMDPFGLVTGLEAVRSPSFEK

SEQ ID NO: 67 - protein, 191 aa, Homo sapiens; identical to SEQ ID NO: 28

SEQ ID NO: 68 - protein, 193 aa, Homo sapiens; identical to SEQ ID NO: 29

SEQ ID NO: 69 - protein, 189 aa, Homo sapiens
RDSSPLVHYGWGDPIRLRHLYTSGPHGLSSCFLRIRADGVVDCARGQSAHSLLEIKAVALRTVAIKGVHSVRYLCMGADGKMQGLLQYSEEDCAFEEEIRPDGYNVYRSEKHRLPVSLSSAKQRQLYKNRGFLPLSHFLPMLPMVPEEPEDLRGHLESDMFSSPLETDSMDPFGLVTGLEAVRSPSFEK

SEQ ID NO: 70 - protein, 190 aa, Homo sapiens
MRDSSPLVHYGWGDPIRLRHLYTSGPHGLSSCFLRIRADGVVDCARGQSAHSLLEIKAVALRTVAIKGVHSVRYLCMGADGKMQGLLQYSEEDCAFEEEIRPDGYNVYRSEKHRLPVSLSSAKQRQLYKNRGFLPLSHFLPMLPMVPEEPEDLRGHLESDMFSSPLETDSMDPFGLVTGLEAVRSPSFEK

SEQ ID NO: 71 - protein, 181 aa, Homo sapiens
HPIPDSSPLLQFGGQVRQRYLYTDDAQQTEAHLEIREDGTVGGAADQSPESLLQLKALKPGVIQILGVKTSRFLCQRPDGALYGSLHFDPEACSFRELLLEDGYNVYQSEAHSLPLHLPGNKSPHRDPAPRGPARFLPLPGLPPALPEPPGILAPQPPDVGSSDPLSMVGPSQGRSPSYAS

SEQ ID NO: 72 - protein, 181 aa, Homo sapiens
HPIPDSSPLLQFGGQVRQRYLYTDDAQQTEAHLEIREDGTVGGAADQSPESLLQLKALKPGVIQILGVKTSRFLCQRPDGALYGSLHFDPEACSFRELLLEDGYNVYQSEAHGLPLHLPGNKSPHRDPAPRGPARFLPLPGLPPAPPEPPGILAPQPPDVGSSDPLSMVGPSQGRSPSYAS

SEQ ID NO: 73 - protein, 212 aa, Homo sapiens
HPIPDSSPLLQFGGQVRQRYLYTDDAQQTEAHLEIREDGTVGGAADQSPESLLQLKALKPGVIQILGVKTSRFLCQRPDGALYGSLHFDPEACSFRELLLEDGYNVYQSEAHGLPLHLPGNKSPHRDPAPRGPARFLPLPGLPPALPEPPGILAPQPPDVGSSDPLSMVVQDELQGVGGEGCHMHPENCKTLLTDIDRTHTEKPVWDGITGE

SEQ ID NO: 74 - protein, 189 aa, Homo sapiens
RDAGPHVHYGWGDPIRLRHLYTSGPHGLSSCFLRIRADGVVDCARGQSAHSLLEIKAVALRTVAIKGVHSVRYLCMGADGKMQGLLQYSEEDCAFEEEIRPDGYNVYRSEKHRLPVSLSSAKQRQLYKNRGFLPLSHFLPMLPMVPEEPEDLRGHLESDMFSSPLETDSMDPFGLVTGLEAVRSPSFEK

SEQ ID NO: 75 - protein, 184 aa, Homo sapiens
RVHYGWGDPIRLRHLYTSGPHGLSSCFLRIRADGVVDCARGQSAHSLLEIKAVALRTVAIKGVHSVRYLCMGADGKMQGLLQYSEEDCAFEEEIRPDGYNVYRSEKHRLPVSLSSAKQRQLYKNRGFLPLSHFLPMLPMVPEEPEDLRGHLESDMFSSPLETDSMDPFGLVTGLEAVRSPSFEK

SEQ ID NO: 76 - protein, 179 aa, Homo sapiens
RGDPIRLRHLYTSGPHGLSSCFLRIRADGVVDCARGQSAHSLLEIKAVALRTVAIKGVHSVRYLCMGADGKMQGLLQYSEEDCAFEEEIRPDGYNVYRSEKHRLPVSLSSAKQRQLYKNRGFLPLSHFLPMLPMVPEEPEDLRGHLESDMFSSPLETDSMDPFGLVTGLEAVRSPSFEK

SEQ ID NO: 77 - protein, 175 aa, Homo sapiens
RRLRHLYTSGPHGLSSCFLRIRADGVVDCARGQSAHSLLEIKAVALRTVAIKGVHSVRYLCMGADGKMQGLLQYSEEDCAFEEEIRPDGYNVYRSEKHRLPVSLSSAKQRQLYKNRGFLPLSHFLPMLPMVPEEPEDLRGHLESDMFSSPLETDSMDPFGLVTGLEAVRSPSFEK

SEQ ID NO: 78 - protein, 188 aa, Homo sapiens
RAGPHVHYGWGDPIRLRHLYTSGPHGLSSCFLRIRADGVVDCARGQSAHSLLEIKAVALRTVAIKGVHSVRYLCMGADGKMQGLLQYSEEDCAFEEEIRPDGYNVYRSEKHRLPVSLSSAKQRQLYKNRGFLPLSHFLPMLPMVPEEPEDLRGHLESDMFSSPLETDSMDPFGLVTGLEAVRSPSFEK

SEQ ID NO: 79 - protein, 187 aa, Homo sapiens
RGPHVHYGWGDPIRLRHLYTSGPHGLSSCFLRIRADGVVDCARGQSAHSLLEIKAVALRTVAIKGVHSVRYLCMGADGKMQGLLQYSEEDCAFEEEIRPDGYNVYRSEKHRLPVSLSSAKQRQLYKNRGFLPLSHFLPMLPMVPEEPEDLRGHLESDMFSSPLETDSMDPFGLVTGLEAVRSPSFEK

SEQ ID NO: 80 - protein, 186 aa, Homo sapiens
RPHVHYGWGDPIRLRHLYTSGPHGLSSCFLRIRADGVVDCARGQSAHSLLEIKAVALRTVAIKGVHSVRYLCMGADGKMQGLLQYSEEDCAFEEEIRPDGYNVYRSEKHRLPVSLSSAKQRQLYKNRGFLPLSHFLPMLPMVPEEPEDLRGHLESDMFSSPLETDSMDPFGLVTGLEAVRSPSFEK

SEQ ID NO: 81 - protein, 185 aa, Homo sapiens
RHVHYGWGDPIRLRHLYTSGPHGLSSCFLRIRADGVVDCARGQSAHSLLEIKAVALRTVAIKGVHSVRYLCMGADGKMQGLLQYSEEDCAFEEEIRPDGYNVYRSEKHRLPVSLSSAKQRQLYKNRGFLPLSHFLPMLPMVPEEPEDLRGHLESDMFSSPLETDSMDPFGLVTGLEAVRSPSFEK

SEQ ID NO: 82 - protein, 194 aa, Homo sapiens
RPLAFSAAGPHVHYGWGDPIRLRHLYTSGPHGLSSCFLRIRADGVVDCARGQSAHSLLEIKAVALRTVAIKGVHSVRYLCMGADGKMQGLLQYSEEDCAFEEEIRPDGYNVYRSEKHRLPVSLSSAKQRQLYKNRGFLPLSHFLPMLPMVPEEPEDLRGHLESDMFSSPLETDSMDPFGLVTGLEAVRSPSFEK

SEQ ID NO: 83 - protein, 194 aa, Homo sapiens
RPLAFSDAAPHVHYGWGDPIRLRHLYTSGPHGLSSCFLRIRADGVVDCARGQSAHSLLEIKAVALRTVAIKGVHSVRYLCMGADGKMQGLLQYSEEDCAFEEEIRPDGYNVYRSEKHRLPVSLSSAKQRQLYKNRGFLPLSHFLPMLPMVPEEPEDLRGHLESDMFSSPLETDSMDPFGLVTGLEAVRSPSFEK

SEQ ID NO: 84 - protein, 194 aa, Homo sapiens
RPLAFSDAGAHVHYGWGDPIRLRHLYTSGPHGLSSCFLRIRADGVVDCARGQSAHSLLEIKAVALRTVAIKGVHSVRYLCMGADGKMQGLLQYSEEDCAFEEEIRPDGYNVYRSEKHRLPVSLSSAKQRQLYKNRGFLPLSHFLPMLPMVPEEPEDLRGHLESDMFSSPLETDSMDPFGLVTGLEAVRSPSFEK

SEQ ID NO: 85 - protein, 194 aa, Homo sapiens
RPLAFSDAGPHVHYGAGDPIRLRHLYTSGPHGLSSCFLRIRADGVVDCARGQSAHSLLEIKAVALRTVAIKGVHSVRYLCMGADGKMQGLLQYSEEDCAFEEEIRPDGYNVYRSEKHRLPVSLSSAKQRQLYKNRGFLPLSHFLPMLPMVPEEPEDLRGHLESDMFSSPLETDSMDPFGLVTGLEAVRSPSFEK

SEQ ID NO: 86 - protein, 194 aa, Homo sapiens
RPLAFSDAGPHVHYGWGAPIRLRHLYTSGPHGLSSCFLRIRADGVVDCARGQSAHSLLEIKAVALRTVAIKGVHSVRYLCMGADGKMQGLLQYSEEDCAFEEEIRPDGYNVYRSEKHRLPVSLSSAKQRQLYKNRGFLPLSHFLPMLPMVPEEPEDLRGHLESDMFSSPLETDSMDPFGLVTGLEAVRSPSFEK

SEQ ID NO: 87 - protein, 167 aa, Homo sapiens
RPLAFSDAGPHVHYGWGDAICARGQSAHSLLEIKAVALRTVAIKGVHSVRYLCMGADGKMQGLLQYSEEDCAFEEEIRPDGYNVYRSEKHRLPVSLSSAKQRQLYKNRGFLPLSHFLPMLPMVPEEPEDLRGHLESDMFSSPLETDSMDPFGLVTGLEAVRSPSFEK

SEQ ID NO: 88 - protein, 194 aa, Homo sapiens
RPLAFSDAGPHVHYGWGDPIRLRHLYTSGPAGLSSCFLRIRADGVVDCARGQSAHSLLEIKAVALRTVAIKGVHSVRYLCMGADGKMQGLLQYSEEDCAFEEEIRPDGYNVYRSEKHRLPVSLSSAKQRQLYKNRGFLPLAHFLPMLPMVPEEPEDLRGHLESDMFSSPLETDSMDPFGLVTGLEAVRSPSFEK

SEQ ID NO: 89 - protein, 194 aa, Homo sapiens
RPLAFSDAGPHVHYGWGDPIRLRHLYTSGPAGLSSCFLRIRADGVVDCARGQSAHSLLEIKAVALRTVAIKGVHSVRYLCMGADGKMQGLLQYSEEDCAFEEEIRPDGYNVYRSEKHRLPVSLSSAKQRQLYKNRGFLPLSAFLPMLPMVPEEPEDLRGHLESDMFSSPLETDSMDPFGLVTGLEAVRSPSFEK

SEQ ID NO: 90 - protein, 194 aa, Homo sapiens
RPLAFSDAGPHVHYGWGDPIRLRHLYTSGPHGLSSCFLRIRADGVVDCARGQSAHSLLEIKAVALRTVAIKGVHSVRYLCMGADGKMQGLLQYSEEDCAFEEEIRPDGYNVYRSEKHRLPVSLSSAAQAQLYKNRGFLPLSHFLPMLPMVPEEPEDLRGHLESDMFSSPLETDSMDPFGLVTGLEAVRSPSFEK

SEQ ID NO: 91 - protein, 194 aa, Homo sapiens
RPLAFSDAGPHVHYGWGDPIRLRHLYTSGPHGLSSCFLRIRADGVVDCARGQSAHSLLEIKAVALRTVAIKGVHSVRYLCMGADGKMQGLLQYSEEDCAFEEEIRPDGYNVYRSEKHRLPVSLSSAAQRQLYKNRGFLPLAHFLPMLPMVPEEPEDLRGHLESDMFSSPLETDSMDPFGLVTGLEAVRSPSFEK

SEQ ID NO: 92 - protein, 194 aa, Homo sapiens
RPLAFSDAGPHVHYGWGDPIRLRHLYTSGPHGLSSCFLRIRADGVVDCARGQSAHSLLEIKAVALRTVAIKGVHSVRYLCMGADGKMQGLLQYSEEDCAFEEEIRPDGYNVYRSEKHRLPVSLSSAAQRQLYKNRGFLPLSAFLPMLPMVPEEPEDLRGHLESDMFSSPLETDSMDPFGLVTGLEAVRSPSFEK

SEQ ID NO: 93 - protein, 194 aa, Homo sapiens
RPLAFSDAGPHVHYGWGDPIRLRHLYTSGPHGLSSCFLRIRADGVVDCARGQSAHSLLEIKAVALRTVAIKGVHSVRYLCMGADGKMQGLLQYSEEDCAFEEEIRPDGYNVYRSEKHRLPVSLSSAKQAQLYKNRGFLPLAHFLPMLPMVPEEPEDLRGHLESDMFSSPLETDSMDPFGLVTGLEAVRSPSFEK

SEQ ID NO: 94 - protein, 194 aa, Homo sapiens
RPLAFSDAGPHVHYGWGDPIRLRHLYTSGPHGLSSCFLRIRADGVVDCARGQSAHSLLEIKAVALRTVAIKGVHSVRYLCMGADGKMQGLLQYSEEDCAFEEEIRPDGYNVYRSEKHRLPVSLSSAKQRQLYKNRGFLPLAAFLPMLPMVPEEPEDLRGHLESDMFSSPLETDSMDPFGLVTGLEAVRSPSFEK

SEQ ID NO: 95 - protein, 194 aa, Homo sapiens; identical to SEQ ID NO: 92

SEQ ID NO: 96 - protein, 194 aa, Homo sapiens
RPLAFSDAGPHVHYGWGDPIRLRHLYTSGPHGLSSCFLRIRADGVVDCARGQSAHSLLEIKAVALRTVAIKGVHSVRYLCMGADGKMQGLLQYSEEDCAFEEEIRPDGYNVYRSEKHRLPVSLSSAAQAQLYKNRGFLPLAHFLPMLPMVPEEPEDLRGHLESDMFSSPLETDSMDPFGLVTGLEAVRSPSFEK

SEQ ID NO: 97 - protein, 194 aa, Homo sapiens
RPLAFSDAGPHVHYGWGDPIRLRHLYTSGPHGLSSCFLRIRADGVVDCARGQSAHSLLEIKAVALRTVAIKGVHSVRYLCMGADGKMQGLLQYSEEDCAFEEEIRPDGYNVYRSEKHRLPVSLSSAAQAQLYKNRGFLPLSAFLPMLPMVPEEPEDLRGHLESDMFSSPLETDSMDPFGLVTGLEAVRSPSFEK

SEQ ID NO: 98 - protein, 194 aa, Homo sapiens
RPLAFSDAGPHVHYGWGDPIRLRHLYTSGPHGLSSCFLRIRADGVVDCARGQSAHSLLEIKAVALRTVAIKGVHSVRYLCMGADGKMQGLLQYSEEDCAFEEEIRPDGYNVYRSEKHRLPVSLSSAAQAQLYKNRGFLPLAAFLPMLPMVPEEPEDLRGHLESDMFSSPLETDSMDPFGLVTGLEAVRSPSFEK

SEQ ID NO: 99 - protein, 194 aa, Homo sapiens
RPLAFSDAGPHVHYGWGDPIRLRHLYTSGPHGLSSCFLRIRADGVVDCARGQSAHSLLEIKAVALRTVAIKGVHSVRYLCMGADGKMQGLLQYSEEDCAFEEEIRPDGYNVYRSEKHRLPVSLSSAKQRQLYKNRGFLPLSHFLPMLPMVPEEPEDLRGHLESDMFSSPLETDSMDPFGLVTGLEAVRSPSFEK

SEQ ID NO: 100 - protein, 181 aa, Homo sapiens
HPIPDSSPLLQFGGQVRQRYLYTDDAQQTEAHLEIREDGTVGGAADQSPESLLQLKALKPGVIQILGVKTSRFLCQRPDGALYGSLHFDPEACSFRELLLEDGYNVYQSEAHGLPLHLPGNKSPHRDPAPRGPARFLPLPGLPPALPEPPGILAPQPPDVGSSDPLSMVGPSQGRSPSYAS

SEQ ID NO: 101 - protein, 4 aa, Homo sapiens
VHYG

SEQ ID NO: 102 - protein, 9 aa, Homo sapiens
DASPHVHYG

SEQ ID NO: 103 - protein, 9 aa, Homo sapiens
DSSPLVHYG

SEQ ID NO: 104 - protein, 7 aa, Homo sapiens
DSSPLLQ

SEQ ID NO: 105 - protein, 12 aa, Homo sapiens
DSSPLLQFGGQV

SEQ ID NO: 106 - protein, 5 aa, Homo sapiens
RHPIP

SEQ ID NO: 107 - protein, 4 aa, Homo sapiens
HPIP

SEQ ID NO: 108 - protein, 5 aa, Homo sapiens
RPLAF

SEQ ID NO: 109 - protein, 4 aa, Homo sapiens
PLAF

SEQ ID NO: 110 - protein, 6 aa, Homo sapiens
MDSSPL

SEQ ID NO: 111 - protein, 7 aa, Homo sapiens
MSDSSPL

SEQ ID NO: 112 - protein, 6 aa, Homo sapiens
SDSSPL

SEQ ID NO: 113 - protein, 5 aa, Homo sapiens
MSSPL

SEQ ID NO: 114 - protein, 4 aa, Homo sapiens
SSPL

SEQ ID NO: 115 - protein, 4 aa, Homo sapiens
RDSS

SEQ ID NO: 116 - protein, 4 aa, Homo sapiens
MDSS

SEQ ID NO: 117 - protein, 5 aa, Homo sapiens
MRDSS

SEQ ID NO: 118 - protein, 5 aa, Homo sapiens
MSSPL

SEQ ID NO: 119 - protein, 6 aa, Homo sapiens
MDSSPL

SEQ ID NO: 120 - protein, 7 aa, Homo sapiens
MSDSSPL

SEQ ID NO: 121 - protein, 5 aa, Homo sapiens
DSSPL

SEQ ID NO: 122 - protein, 5 aa, Homo sapiens
DASPH

SEQ ID NO: 123 - protein, 4 aa, Homo sapiens
RDSS

SEQ ID NO: 124 - protein, 4 aa, Homo sapiens
MDSS

SEQ ID NO: 125 - protein, 5 aa, Homo sapiens
MRDSS

SEQ ID NO: 126 - protein, 6 aa, Homo sapiens
MDSSPL

SEQ ID NO: 127 - protein, 7 aa, Homo sapiens
MSDSSPL

SEQ ID NO: 128 - protein, 5 aa, Homo sapiens
MSSPL

SEQ ID NO: 129 - protein, 5 aa, Artificial Sequence
  Description of Artificial Sequence: Linker sequence
GSGGS

SEQ ID NO: 130 - protein, 4 aa, Artificial Sequence
  Description of Artificial Sequence: Linker sequence
GGGS

SEQ ID NO: 131 - protein, 4 aa, Artificial Sequence
  Description of Artificial Sequence: Linker sequence
GGSG

SEQ ID NO: 132 - protein, 5 aa, Artificial Sequence
  Description of Artificial Sequence: Linker sequence
GGSGG

SEQ ID NO: 133 - protein, 5 aa, Artificial Sequence
  Description of Artificial Sequence: Linker sequence
GSGSG

SEQ ID NO: 134 - protein, 5 aa, Artificial Sequence
  Description of Artificial Sequence: Linker sequence
GSGGG

SEQ ID NO: 135 - protein, 5 aa, Artificial Sequence
  Description of Artificial Sequence: Linker sequence
GSSSG

SEQ ID NO: 136 - DNA, 32 bp, Artificial Sequence
  Description of Artificial Sequence: Forward primer
ccgactagtcaccatgcggagcgggtgtgtgg

SEQ ID NO: 137 - DNA, 41 bp, Artificial Sequence
  Description of Artificial Sequence: Reverse primer
ataagaatgcggccgcttacttctcaaagctgggactcctc

SEQ ID NO: 138 - protein, 186 aa, Homo sapiens
DSSPLLQFGGQVRLRHLYTSGPHGLSSCFLRIRADGVVDCARGQSAHSLLEIKAVALRTVAIKGVHSVRYLCMGADGKMQGLLQYSEEDCAFEEEIRPDGYNVYRSEKHRLPVSLSSAKQRQLYKNRGFLPLSHFLPMLPMVPEEPEDLRGHLESDMFSSPLETDSMDPFGLVTGLEAVRSPSFEK

SEQ ID NO: 139 - protein, 194 aa, Homo sapiens; identical to SEQ ID NO: 1

SEQ ID NO: 140 - protein, 194 aa, Homo sapiens; identical to SEQ ID NO: 2

SEQ ID NO: 141 - protein, 188 aa, Homo sapiens
DSSPLVHYGWGDPIRLRHLYTSGPHGLSSCFLRIRADGVVDCARGQSAHSLLEIKAVALRTVAIKGVHSVRYLCMGADGKMQGLLQYSEEDCAFEEEIRPDGYNVYRSEKHRLPVSLSSAKQRQLYKNRGFLPLSHFLPMLPMVPEEPEDLRGHLESDMFSSPLETDSMDPFGLVTGLEAVRSPSFEK

SEQ ID NO: 142 - protein, 193 aa, Homo sapiens; identical to SEQ ID NO: 9

SEQ ID NO: 143 - protein, 191 aa, Homo sapiens; identical to SEQ ID NO: 8

SEQ ID NO: 144 - protein, 194 aa, Homo sapiens; identical to SEQ ID NO: 12

SEQ ID NO: 145 - protein, 193 aa, Homo sapiens; identical to SEQ ID NO: 10

SEQ ID NO: 146 - protein, 192 aa, Homo sapiens; identical to SEQ ID NO: 13

SEQ ID NO: 147 - protein, 191 aa, Homo sapiens; identical to SEQ ID NO: 14

SEQ ID NO: 148 - protein, 187 aa, Homo sapiens; identical to SEQ ID NO: 6

SEQ ID NO: 149 - protein, 192 aa, Homo sapiens; identical to SEQ ID NO: 7

SEQ ID NO: 150 - protein, 191 aa, Homo sapiens; identical to SEQ ID NO: 31

SEQ ID NO: 151 - protein, 191 aa, Homo sapiens; identical to SEQ ID NO: 32

SEQ ID NO: 152 - protein, 191 aa, Homo sapiens; identical to SEQ ID NO: 33

SEQ ID NO: 153 - protein, 191 aa, Homo sapiens; identical to SEQ ID NO: 34

SEQ ID NO: 154 - protein, 191 aa, Homo sapiens; identical to SEQ ID NO: 35

SEQ ID NO: 155 - protein, 191 aa, Homo sapiens; identical to SEQ ID NO: 36

SEQ ID NO: 156 - protein, 191 aa, Homo sapiens; identical to SEQ ID NO: 37

SEQ ID NO: 157 - protein, 191 aa, Homo sapiens; identical to SEQ ID NO: 38

SEQ ID NO: 158 - protein, 191 aa, Homo sapiens; identical to SEQ ID NO: 39

SEQ ID NO: 159 - protein, 193 aa, Homo sapiens; identical to SEQ ID NO: 40

SEQ ID NO: 160 - protein, 190 aa, Homo sapiens
HPIPDSSPLLQFGGQVRLRHLYTSGPHGLSSCFLRIRADGVVDCARGQSAHSLLEIKAVALRTVAIKGVHSVRYLCMGADGKMQGLLQYSEEDCAFEEEIRPDGYNVYRSEKHRLPVSLSSAKQRQLYKNRGFLPLSHFLPMLPMVPEEPEDLRGHLESDMFSSPLETDSMDPFGLVTGLEAVRSPSFEK

SEQ ID NO: 161 - protein, 186 aa, Homo sapiens; identical to SEQ ID NO: 138

SEQ ID NO: 162 - protein, 190 aa, Homo sapiens; identical to SEQ ID NO: 47

SEQ ID NO: 163 - protein, 192 aa, Homo sapiens
HPIPDSSPLLQFGWGDPIRLRHLYTSGPHGLSSCFLRIRADGVVDCARGQSAHSLLEIKAVALRTVAIKGVHSVRYLCMGADGKMQGLLQYSEEDCAFEEEIRPDGYNVYRSEKHRLPVSLSSAKQRQLYKNRGFLPLSHFLPMLPMVPEEPEDLRGHLESDMFSSPLETDSMDPFGLVTGLEAVRSPSFEK

SEQ ID NO: 164 - protein, 192 aa, Homo sapiens
HPIPDSSPHVHYGWGDPIRLRHLYTSGPHGLSSCFLRIRADGVVDCARGQSAHSLLEIKAVALRTVAIKGVHSVRYLCMGADGKMQGLLQYSEEDCAFEEEIRPDGYNVYRSEKHRLPVSLSSAKQRQLYKNRGFLPLSHFLPMLPMVPEEPEDLRGHLESDMFSSPLETDSMDPFGLVTGLEAVRSPSFEK

SEQ ID NO: 165 - protein, 190 aa, Homo sapiens
HPIPDSSPHVHYGGQVRLRHLYTSGPHGLSSCFLRIRADGVVDCARGQSAHSLLEIKAVALRTVAIKGVHSVRYLCMGADGKMQGLLQYSEEDCAFEEEIRPDGYNVYRSEKHRLPVSLSSAKQRQLYKNRGFLPLSHFLPMLPMVPEEPEDLRGHLESDMFSSPLETDSMDPFGLVTGLEAVRSPSFEK

SEQ ID NO: 166 - protein, 188 aa, Homo sapiens
DAGPHVHYGWGDPIRLRHLYTSGPHGLSSCFLRIRADGVVDCARGQSAHSLLEIKAVALRTVAIKGVHSVRYLCMGADGKMQGLLQYSEEDCAFEEEIRPDGYNVYRSEKHRLPVSLSSAKQRQLYKNRGFLPLSHFLPMLPMVPEEPEDLRGHLESDMFSSPLETDSMDPFGLVTGLEAVRSPSFEK

SEQ ID NO: 167 - protein, 183 aa, Homo sapiens
VHYGWGDPIRLRHLYTSGPHGLSSCFLRIRADGVVDCARGQSAHSLLEIKAVALRTVAIKGVHSVRYLCMGADGKMQGLLQYSEEDCAFEEEIRPDGYNVYRSEKHRLPVSLSSAKQRQLYKNRGFLPLSHFLPMLPMVPEEPEDLRGHLESDMFSSPLETDSMDPFGLVTGLEAVRSPSFEK

SEQ ID NO: 168 - protein, 174 aa, Homo sapiens
RLRHLYTSGPHGLSSCFLRIRADGVVDCARGQSAHSLLEIKAVALRTVAIKGVHSVRYLCMGADGKMQGLLQYSEEDCAFEEEIRPDGYNVYRSEKHRLPVSLSSAKQRQLYKNRGFLPLSHFLPMLPMVPEEPEDLRGHLESDMFSSPLETDSMDPFGLVTGLEAVRSPSFEK

SEQ ID NO: 169 - protein, 14 aa, Artificial Sequence
  Synthetic peptide
WGDPIRLRHLYTSG

SEQ ID NO: 170 - protein, 5 aa, Artificial Sequence
  Synthetic peptide
WGDPI

SEQ ID NO: 171 - protein, 4 aa, Artificial Sequence
  Synthetic peptide
WGPI

SEQ ID NO: 172 - protein, 5 aa, Artificial Sequence
  Synthetic peptide
WGDPV

SEQ ID NO: 173 - protein, 4 aa, Artificial Sequence
  Synthetic peptide
WGDI

SEQ ID NO: 174 - protein, 4 aa, Artificial Sequence
  Synthetic peptide
GDPI

SEQ ID NO: 175 - protein, 5 aa, Artificial Sequence
  Synthetic peptide
WGQPI

SEQ ID NO: 176 - protein, 5 aa, Artificial Sequence
  Synthetic peptide
WGAPI

SEQ ID NO: 177 - protein, 5 aa, Artificial Sequence
  Synthetic peptide
AGDPI

SEQ ID NO: 178 - protein, 5 aa, Artificial Sequence
  Synthetic peptide
WADPI

SEQ ID NO: 179 - protein, 5 aa, Artificial Sequence
  Synthetic peptide
WGDAI

SEQ ID NO: 180 - protein, 5 aa, Artificial Sequence
  Synthetic peptide
WGDPA

SEQ ID NO: 181 - protein, 4 aa, Artificial Sequence
  Synthetic peptide
WDPI

SEQ ID NO: 182 - protein, 4 aa, Artificial Sequence
  Synthetic peptide
WGDI

SEQ ID NO: 183 - protein, 4 aa, Artificial Sequence
  Synthetic peptide
WGDP

SEQ ID NO: 184 - protein, 5 aa, Artificial Sequence
  Synthetic peptide
FGDPI

SEQ ID NO: 185 - protein, 9 aa, Artificial Sequence
  Synthetic peptide
RLRHLYTSG

SEQ ID NO: 186 - protein, 9 aa, Artificial Sequence
  core sequence
RQRYLYTDD

SEQ ID NO: 187 - protein, 13 aa, Artificial Sequence
  Synthetic peptide
AGPHVHYGWGDPI

SEQ ID NO: 188 - protein, 165 aa, Homo sapiens
  FGF19 C-terminal sequence
PHGLSSCFLRIRADGVVDCARGQSAHSLLEIKAVALRTVAIKGVHSVRYLCMGADGKMQGLLQYSEEDCAFEEEIRPDGYNVYRSEKHRLPVSLSSAKQRQLYKNRGFLPLSHFLPMLPMVPEEPEDLRGHLESDMFSSPLETDSMDPFGLVTGLEAVRSPSFEK

SEQ ID NO: 189 - protein, 5 aa, Artificial Sequence
  Linker sequence
GGGSG

SEQ ID NO: 190 - protein, 11 aa, Homo sapiens
  Sheet-8/Loop-8/Sheet-9 region of FGF19
EEIRPDGYNVY

SEQ ID NO: 191 - protein, 11 aa, Homo sapiens
  Sheet-8/Loop-8/Sheet-9 region of FGF21
ELLLEDGYNVY

SEQ ID NO: 192 - protein, 187 aa, Artificial Sequence
  M53 sequence
MDSSPLLQWGDPIRLRHLYTSGPHGLSSCFLRIRADGVVDCARGQSAHSLLEIKAVALRTVAIKGVHSVRYLCMGADGKMQGLLQYSEEDCAFEEEIRPDGYNVYRSEKHRLPVSLSSAKQRQLYKNRGFLPLSHFLPMLPMVPEEPEDLRGHLESDMFSSPLETDSMDPFGLVTGLEAVRSPSFEK

SEQ ID NO: 193 - protein, 194 aa, Artificial Sequence
  M139 sequence
RPLAFSDAGPHVHYGWGDPIRLRHLYTSGPHGLSSCFLRIRADGVVDCARGQSAHSLLEIKAVALRTVAIKGVHSVRYLCMGADGKMQGLLQYSEEDCAFEEEILPDGYNVYRSEKHRLPVSLSSAKQRQLYKNRGFLPLSHFLPMLPMVPEEPEDLRGHLESDMFSSPLETDSMDPFGLVTGLEAVRSPSFEK

SEQ ID NO: 194 - protein, 194 aa, Artificial Sequence
  M140 sequence
RPLAFSDAGPHVHYGWGDPIRLRHLYTSGPHGLSSCFLRIRADGVVDCARGQSAHSLLEIKAVALRTVAIKGVHSVRYLCMGADGKMQGLLQYSEEDCAFEEEIREDGYNVYRSEKHRLPVSLSSAKQRQLYKNRGFLPLSHFLPMLPMVPEEPEDLRGHLESDMFSSPLETDSMDPFGLVTGLEAVRSPSFEK

SEQ ID NO: 195 - protein, 194 aa, Artificial Sequence
  M141 sequence
RPLAFSDAGPHVHYGWGDPIRLRHLYTSGPHGLSSCFLRIRADGVVDCARGQSAHSLLEIKAVALRTVAIKGVHSVRYLCMGADGKMQGLLQYSEEDCAFEEEILCDGYNVYRSEKHRLPVSLSSAKQRQLYKNRGFLPLSHFLPMLPMVPEEPEDLRGHLESDMFSSPLETDSMDPFGLVTGLEAVRSPSFEK

SEQ ID NO: 196 - protein, 194 aa, Artificial Sequence
  M160 sequence
RPLAFSDAGPHVHYGWGDPIRQRHLYTSGPHGLSSCFLRIRADGVVDCARGQSAHSLLEIKAVALRTVAIKGVHSVRYLCMGADGKMQGLLQYSEEDCAFEEEILEDGYNVYRSEKHRLPVSLSSAKQRQLYKNRGFLPLSHFLPMLPMVPEEPEDLRGHLESDMFSSPLETDSMDPFGLVTGLEAVRSPSFEK

SEQ ID NO: 197 - protein, 189 aa, Artificial Sequence
  M200 Sequence
RDSSPLVHYGWGDPIRLRHLYTSGPHGLSSCFLRIRADGVVDCARGQSAHSLLEIKAVALRTVAIKGVHSVRYLCMGADGKMQGLLQYSEEDCAFEEEILEDGYNVYRSEKHRLPVSLSSAKQRQLYKNRGFLPLSHFLPMLPMVPEEPEDLRGHLESDMFSSPLETDSMDPFGLVTGLEAVRSPSFEK

SEQ ID NO: 198 - protein, 194 aa, Artificial Sequence
  M201 Sequence
RPLAFSDSSPLVHYGWGDPIRLRHLYTSGPHGLSSCFLRIRADGVVDCARGQSAHSLLEIKAVALRTVAIKGVHSVRYLCMGADGKMQGLLQYSEEDCAFEEEILEDGYNVYRSEKHRLPVSLSSAKQRQLYKNRGFLPLSHFLPMLPMVPEEPEDLRGHLESDMFSSPLETDSMDPFGLVTGLEAVRSPSFEK

SEQ ID NO: 199 - protein, 194 aa, Artificial Sequence
  M202 Sequence
RPLAFSDASPHVHYGWGDPIRLRHLYTSGPHGLSSCFLRIRADGVVDCARGQSAHSLLEIKAVALRTVAIKGVHSVRYLCMGADGKMQGLLQYSEEDCAFEEEILEDGYNVYRSEKHRLPVSLSSAKQRQLYKNRGFLPLSHFLPMLPMVPEEPEDLRGHLESDMFSSPLETDSMDPFGLVTGLEAVRSPSFEK

SEQ ID NO: 200 - protein, 187 aa, Artificial Sequence
  M203 Sequence
RDSSPLLQWGDPIRLRHLYTSGPHGLSSCFLRIRADGVVDCARGQSAHSLLEIKAVALRTVAIKGVHSVRYLCMGADGKMQGLLQYSEEDCAFEEEILEDGYNVYRSEKHRLPVSLSSAKQRQLYKNRGFLPLSHFLPMLPMVPEEPEDLRGHLESDMFSSPLETDSMDPFGLVTGLEAVRSPSFEK

SEQ ID NO: 201 - protein, 191 aa, Artificial Sequence; identical to SEQ ID NO: 50
  M204 Sequence

SEQ ID NO: 202 - protein, 187 aa, Artificial Sequence
  M205 Sequence
RDSSPLLQFGGQVRLRHLYTSGPHGLSSCFLRIRADGVVDCARGQSAHSLLEIKAVALRTVAIKGVHSVRYLCMGADGKMQGLLQYSEEDCAFEEEILEDGYNVYRSEKHRLPVSLSSAKQRQLYKNRGFLPLSHFLPMLPMVPEEPEDLRGHLESDMFSSPLETDSMDPFGLVTGLEAVRSPSFEK

SEQ ID NO: 203 - protein, 191 aa, Artificial Sequence
  M206 Sequence
RHPIPDSSPLLQFGGQVRLRHLYTSGPHGLSSCFLRIRADGVVDCARGQSAHSLLEIKAVALRTVAIKGVHSVRYLCMGADGKMQGLLQYSEEDCAFEEEILEDGYNVYRSEKHRLPVSLSSAKQRQLYKNRGFLPLSHFLPMLPMVPEEPEDLRGHLESDMFSSPLETDSMDPFGLVTGLEAVRSPSFEK

SEQ ID NO: 204 - protein, 190 aa, Artificial Sequence
  M207 Sequence
MRDSSPLVHYGWGDPIRLRHLYTSGPHGLSSCFLRIRADGVVDCARGQSAHSLLEIKAVALRTVAIKGVHSVRYLCMGADGKMQGLLQYSEEDCAFEEEILEDGYNVYRSEKHRLPVSLSSAKQRQLYKNRGFLPLSHFLPMLPMVPEEPEDLRGHLESDMFSSPLETDSMDPFGLVTGLEAVRSPSFEK

SEQ ID NO: 205 - protein, 11 aa, Artificial Sequence
  Modified Sheet-8/Loop-8/Sheet-9 region of FGF19
EEILEDGYNVY